European Patent Application EP 4 737 576 A1, published May 6, 2026. Title: 一种高效获得肿瘤抗原特异性B细胞的小鼠模型的构建和应用. Applicant: 北京干细胞与再生医学研究院. The sequence listing filed with the application follows.

SEQUENCE LISTING (16 sequences)

SEQ ID NO: 1 - DNA, 2598 bp, synthetic construct
  source 1..2598: mol_type = other DNA
ggaagcggagagggaaggggctccctgctgacctgtggcgacgtggaggagaaccccggaccaatggctctgccagtgacagccctgctgctgccactggccctgctgctgcacgctgctaggccagagcagaagctgatctccgaggaggatctgatggctcaggtgcagctggtggagtctggcggacgcctggtgcaggctggcgactccctgagactgtcttgcgccgctagcggacggaccttcagcacatccgctatggcctggtttaggcaggctccaggaagagagagggagttcgtggccgctatcacctggacagtgggaaataccatcctgggcgattccgtgaagggcaggttcaccatcagccgcgacagggccaagaacacagtggacctgcagatggataatctggagccagaggacacagccgtgtactattgttccgccagatctcggggctacgtgctgtccgtgctgagaagcgtggactcctacgattattggggacagggcacccaggtgacagtgagcggcggaggaggcagcggaggaggaggatctggcggaggcggaagcatggcccaggtccagctggtggagagcggaggaggactggtgcaggctggaggctccctgaggctgtcttgcgctgctagcggcaggaccttctccaactacgctatgggctggtttcgccaggcccctggaaaggaaagagaatttgtggccgctatctcctggaccggcgtgtctacatactatgccgattctgtcaaaggcaggttcaccatcagcagagacaacgataagaatacagtgtatgtgcagatgaactccctgatccccgaggacaccgctatctactattgtgccgctgtgcgcgccaggtctttcagcgatacatactctcgggtgaatgagtacgactactggggccagggtacacaggtgacagtgatcctggattatagctttaccggaggagctggaagggacatccctccaccacagatcgaggaggcttgcgagctgccagagtgtcaggtggacgctggcaacaaggtgtgcaatctgcagtgtaacaatcacgcctgcggatgggacggaggcgattgtagcctgaacttcaatgacccatggaagaactgcacccagtctctgcagtgttggaagtactttagcgacggccactgcgattcccagtgtaactctgccggctgcctgttcgacggatttgattgtcagctgacagagggccagtgcaatcctctgtacgaccagtattgcaaggaccacttctctgatggccactgcgaccagggatgtaacagcgccgagtgtgagtgggacggcctggattgcgctgagcacgtgccagagcggctggctgctggaaccctggtgctggtggtgctgctgcctccagatcagctgagaaacaattccttccactttctgcgggagctgtctcacgtgctgcacacaaatgtggtgttcaagagagacgctcagggccagcagatgatctttccttactatggacacgaggaggagctgagaaagcaccccatcaagcggtccaccgtgggatgggccacaagctccctgctgccaggaacctctggaggccgccagaggagagagctggaccctatggacatcaggggctccatcgtgtacctggagatcgataacagacagtgcgtgcagtctagctcccagtgcttccagtctgctacagacgtggccgcttttctgggcgctctggcctctctgggaagcctgaatatcccatacaagatcgaggccgtgaagagcgagcctgtggagccacctctgccatcccagctgcacctgatgtatgtggccgctgccgctttcgtgctgctgttctttgtgggatgtggcgtgctgctgtccaggaagcggcgcaggcagctgtgcatccagaagctgatgaagctgctgtctagcatcgagcaggcttgcgacatctgtaggctgaagaagctgaagtgtagcaaggagaagcctaagtgcgccaagtgtctgaagaacaattgggagtgcagatattctccaaagaccaagcgcagccctctgaccagggctcacctgacagaggtggagtctagactggagcggctggagcagctgttcctgctgatctttccaagagaggacctggatatgatcctgaagatggatagcctgcaggacatcaaggccctgctgaccggcctgttcgtgcaggataacgtgaataaggatgctgtgacagacaggctggctagcgtggagaccgacatgcctctgacactgcgccagcacaggatctccgccacctcctctagcgaggagtcctctaacaagggacagaggcagctgacagtgagcgccgctgccggaggctccggaggctctggaggcagcgatgctctggacgatttcgacctggatatgctgggcagcgacgccctggacgattttgacctggacatgctcggcagcgacgcactcgatgactttgacctggacatgctgggctctgatgctctcgatgattttgacctggatatgctgggaagc

SEQ ID NO: 2 - DNA, 870 bp, synthetic construct
  source 1..870: mol_type = other DNA
atgcataaggagcactgtcctccgaacgggagcactgtcctccgaacgggagcactgtcctccgaacgggagcactgtcctccgaacgggagcactgtcctccgaacgggtaggcgtgtacggtgggaggcctatataagcagagctgaattcatggtgagcaagggcgaggaggataacatggccatcatcaaggagttcatgcgcttcaaggtgcacatggagggctccgtgaacggccacgagttcgagatcgagggcgagggcgagggccgcccctacgagggcacccagaccgccaagctgaaggtgaccaagggtggccccctgcccttcgcctgggacatcctgtcccctcagttcatgtacggctccaaggcctacgtgaagcaccccgccgacatccccgactacttgaagctgtccttccccgagggcttcaagtgggagcgcgtgatgaacttcgaggacggcggcgtggtgaccgtgacccaggactcctccctgcaggacggcgagttcatctacaaggtgaagctgcgcggcaccaacttcccctccgacggccccgtaatgcagaagaagaccatgggctgggaggcctcctccgagcggatgtaccccgaggacggcgccctgaagggcgagatcaagcagaggctgaagctgaaggacggcggccactacgacgctgaggtcaagaccacctacaaggccaagaagcccgtgcagctgcccggcgcctacaacgtcaacatcaagttggacatcacctcccacaacgaggactacaccatcgtggaacagtacgaacgcgccgagggccgccactccaccggcggcatggacgagctgtacaagtgagctagc

SEQ ID NO: 3 - DNA, 1113 bp, synthetic construct
  source 1..1113: mol_type = other DNA
gcttgggtgttgatgttcccgcctttgcctgcctgtccgctctggtcctcatcactggtgagtggcagaaactagactgggcccaagggttgcaggaccattgggtaggtagcatctaacactttggggacccctagagtgcctgcaacattgggatgttaggacctgcaaagggacttagctctattcgcccctaaagcttaaatcagcctccgaatgaccccggactcctcaggtacgactgtaggcgctgggcatctagcttagggattctgtttgtttaaaaacctagctgtcaacctcacaagacacaggaacgtgcacacatgaatttttcacattctgcgcttggatagctatcgccatggtccagaaacaggacctacttcagctctgttgggctccctccttattgtctctgtaagaggtaaccactctgccagcctcagtggcattcctgtcatggattttactgtgcgtatcacagggtatggactctagtgttaaatgtagaggtttctgggtcccttctgcttccgctcccatttccacttaaatttcttaggggatcctcctgagtagatcaagaccaggagctggatcttgaaagggtagggagtgatatctacacccagctcgtccttagtctgtcctgcgagactccaggattttagaacagtgtggagcctggacctccagaaaacctggattaggcttttgccttggccagccattcagtggtttcaaatattgaccagtctggacagtgggctcctgtgggacgtgctagagggctggggaagcttgtcagggagaaggcgtcaactgagcggggctgactctaccttccctgctgcagatcgacacgggctccaggaccctcgtcgggtggaagagctgcagaatcgcattgctagctgtctgaaggagcacatggctaccgtggcaggagacccacagccggccagctgcctgtcacgtctgctgggcaaactgcctgagcttcggaccctgtgcactcaaggcctgcagcgcatcttttgcctcaagttggaggacttggtaccccctccacctattgtggacaagatctttatggacacattgtctttc

SEQ ID NO: 4 - DNA, 1168 bp, synthetic construct
  source 1..1168: mol_type = other DNA
cccctgccctgaacatgtgtgcgcacacgtgcgtgctcttctgtcacccatgtgcctttaagcctatagcccacggacccccagaccaccctacccccagcctggttttgagctaagactgacgtacctcctcactccagaagatggacagagaactcaagacctgggggagggtgtgtattcacgggggtgaccccactatttgtcttatccctccagctcagtcctggccttcgtgtgtttttgtaagataaaccatttttaacacataccactctgttgtaaataagctgacgctactgtaaatacagaaaggaagaggttgagatgggggttgggaggaaggggtggggctcccaccagctgggcgagcctccaactcgagatctcttccgctctccttccatgtgtacataactgtcactcaagaaggtgattgacagattctgatttatatttgtgtattttcctggatttataggatgtgacttttctgattaatatatttaatatattgaataaaaaatagacatgtagttgaaattgagtctttttttctgtttttgttttttgtttttttttttttgtttttgtttttgtttttttgttttgtttttcgagacagggtttctctgtatagccctggctgtcctggagctcactttgtagaccaggctggcctcgaactcagaaatccgcctgcctctgcctcccgagtgctgggattaaaggcgtgcaccaccatgcctggctttttctgacagcactagacattttgccatgattatataagagacagcagtagccctgggcaaatcttagctgttgccagtgatctggtcagcctgggttacttacctgtaggtgataggtcatgatgaagcctgcttcatgcagccatttaggagaactctgggactagcttgcctttctcacacaaacacctgtctcaccatggtgcccggatggtttagacttgctgtgtagcttggctagtttcaagctgtcagtcttcctatctccacttcctgagtgttgggattatagatgttcaccctacacatgcatcgggagctagttcctaatgtgggaagcctctggttaccgctggctgccagacctcagtggacagcggctaacccagggactagagcagcaagatagacct

SEQ ID NO: 5 - DNA, 822 bp, synthetic construct
  source 1..822: mol_type = other DNA
aatggcgtgttttggttggcgtaaggcgcctgtcagttaacggcagccggagtgcgcagccgccggcagcctcgctctgcccactgggtggggcgggaggtaggtggggtgaggcgagctggacgtgcgggcgcggtcggcctctggcggggcgggggaggggagggagggtcagcgaaagtagctcgcgcgcgagcggccgcccaccctccccttcctctgggggagtcgttttacccgccgccggccgggcctcgtcgtctgattggctctcggggcccagaaaactggcccttgccattggctcgtgttcgtgcaagttgagtccatccgccggccagcgggggcggcgaggaggcgctcccaggttccggccctcccctcggccccgcgccgcagagtctggccgcgcgcccctgcgcaacgtggcaggaagcgcgcgctgggggcggggacgggcagtagggctgagcggctgcggggcgggtgcaagcacgtttccgacttgagttgcctcaagaggggcgtgctgagccagacctccatcgcgcactccggggagtggagggaaggagcgagggctcagttgggctgttttggaggcaggaagcacttgctctcccaaagtcgctctgagttgttatcagtaagggagctgcagtggagtaggcggggagaaggccgcacccttctccggaggggggaggggagtgttgcaatacctttctgggagttctctgctgcctcctggcttctgaggaccgccctgggcctgggagaatcccttccccctcttccctcgtgatctgcaactccagtctt

SEQ ID NO: 6 - DNA, 849 bp, synthetic construct
  source 1..849: mol_type = other DNA
agatgggcgggagtcttctgggcaggcttaaaggctaacctggtgtgtgggcgttgtcctgcaggggaattgaacaggtgtaaaattggagggacaagacttcccacagattttcggttttgtcgggaagttttttaataggggcaaataaggaaaatgggaggataggtagtcatctggggttttatgcagcaaaactacaggttattattgcttgtgatccgcctcggagtattttccatcgaggtagattaaagacatgctcacccgagttttatactctcctgcttgagatccttactacagtatgaaattacagtgtcgcgagttagactatgtaagcagaattttaatcatttttaaagagcccagtacttcatatccatttctcccgctccttctgcagccttatcaaaaggtattttagaacactcattttagccccattttcatttattatactggcttatccaacccctagacagagcattggcattttccctttcctgatcttagaagtctgatgactcatgaaaccagacagattagttacatacaccacaaatcgaggctgtagctggggcctcaacactgcagttcttttataactccttagtacactttttgttgatcctttgccttgatccttaattttcagtgtctatcacctctcccgtcaggtggtgttccacatttgggcctattctcagtccagggagttttacaacaatagatgtattgagaatccaacctaaagcttaactttccactcccatgaatgcctctctcctttttctccatttataaactgagctattaaccattaatggtttccaggtggatgtctcc

SEQ ID NO: 7 - DNA, 20 bp, synthetic construct
  source 1..20: mol_type = other DNA
gctccaggaccctcgtcggg

SEQ ID NO: 8 - DNA, 20 bp, synthetic construct
  source 1..20: mol_type = other DNA
gggccgcacccttctccgga

SEQ ID NO: 9 - protein, 310 aa, synthetic construct
METDTLLLWVLLLWVPGSTGDMVSKGEELFTGVVPILVELDGDVNGHKFSVSGEGEGDATYGKLTLKFICTTGKLPVPWPTLVTTLTYGVQCFSRYPDHMKQHDFFKSAMPEGYVQERTIFFKDDGNYKTRAEVKFEGDTLVNRIELKGIDFKEDGNILGHKLEYNYNSHNVYIMADKQKNGIKVNFKIRHNIEDGSVQLADHYQQNTPIGDGPVLLPDNHYLSTQSALSKDPNEKRDHMVLLEFVTAAGITLGMDELYKNAVGQDTQEVIVVPHSLPFKVVVISAILALVVLTIISLIILIMLWQKKPR

SEQ ID NO: 10 - protein, 370 aa, synthetic construct
METDTLLLWVLLLWVPGSTGDYPYDVPDYAGAQPARPEEPLVVKVEEGDNAVLQCLKGTSDGPTQQLTWSRESPLKPFLKLSLGLPGLGIHMRPLAIWLFIFNVSQQMGGFYLCQPGPPSEKAWQPGWTVNVEGSGELFRWNVSDLGGLGCGLKNRSSEGPSSPSGKLMSPKLYVWAKDRPEIWEGEPPCLPPRDSLNQSLSQDLTMAPGSTLWLSCGVPPDSVSRGPLSWTHVHPKGPKSLLSLELKDDRPARDMWVMETGLLLPRATAQDAGKYYCHRGNLTMSFHLEITARPVLWHWLLRTGGWKVDEQKLISEEDLNAVGQDTQEVIVVPHSLPFKVVVISAILALVVLTIISLIILIMLWQKKPR

SEQ ID NO: 11 - DNA, 7798 bp, synthetic construct
  source 1..7798: mol_type = other DNA
ctaaattgtaagcgttaatattttgttaaaattcgcgttaaatttttgttaaatcagctcattttttaaccaataggccgaaatcggcaaaatcccttataaatcaaaagaatagaccgagatagggttgagtgttgttccagtttggaacaagagtccactattaaagaacgtggactccaacgtcaaagggcgaaaaaccgtctatcagggcgatggcccactacgtgaaccatcaccctaatcaagttttttggggtcgaggtgccgtaaagcactaaatcggaaccctaaagggagcccccgatttagagcttgacggggaaagccggcgaacgtggcgagaaaggaagggaagaaagcgaaaggagcgggcgctagggcgctggcaagtgtagcggtcacgctgcgcgtaaccaccacacccgccgcgcttaatgcgccgctacagggcgcgtcccattcgccattcaggctgcgcaactgttgggaagggcgatcggtgcgggcctcttcgctattacgccagctggcgaaagggggatgtgctgcaaggcgattaagttgggtaacgccagggttttcccagtcacgacgttgtaaaacgacggccagtgagcgcgcgtaatacgactcactatagggcgaattgggtaccgggccccccctcgaggtcgacgcttgggtgttgatgttcccgcctttgcctgcctgtccgctctggtcctcatcactggtgagtggcagaaactagactgggcccaagggttgcaggaccattgggtaggtagcatctaacactttggggacccctagagtgcctgcaacattgggatgttaggacctgcaaagggacttagctctattcgcccctaaagcttaaatcagcctccgaatgaccccggactcctcaggtacgactgtaggcgctgggcatctagcttagggattctgtttgtttaaaaacctagctgtcaacctcacaagacacaggaacgtgcacacatgaatttttcacattctgcgcttggatagctatcgccatggtccagaaacaggacctacttcagctctgttgggctccctccttattgtctctgtaagaggtaaccactctgccagcctcagtggcattcctgtcatggattttactgtgcgtatcacagggtatggactctagtgttaaatgtagaggtttctgggtcccttctgcttccgctcccatttccacttaaatttcttaggggatcctcctgagtagatcaagaccaggagctggatcttgaaagggtagggagtgatatctacacccagctcgtccttagtctgtcctgcgagactccaggattttagaacagtgtggagcctggacctccagaaaacctggattaggcttttgccttggccagccattcagtggtttcaaatattgaccagtctggacagtgggctcctgtgggacgtgctagagggctggggaagcttgtcagggagaaggcgtcaactgagcggggctgactctaccttccctgctgcagatcgacacgggctccaggaccctcgtcgggtggaagagctgcagaatcgcattgctagctgtctgaaggagcacatggctaccgtggcaggagacccacagccggccagctgcctgtcacgtctgctgggcaaactgcctgagcttcggaccctgtgcactcaaggcctgcagcgcatcttttgcctcaagttggaggacttggtaccccctccacctattgtggacaagatctttatggacacattgtctttcgatatcggaagcggagagggaaggggctccctgctgacctgtggcgacgtggaggagaaccccggaccaatggctctgccagtgacagccctgctgctgccactggccctgctgctgcacgctgctaggccagagcagaagctgatctccgaggaggatctgatggctcaggtgcagctggtggagtctggcggacgcctggtgcaggctggcgactccctgagactgtcttgcgccgctagcggacggaccttcagcacatccgctatggcctggtttaggcaggctccaggaagagagagggagttcgtggccgctatcacctggacagtgggaaataccatcctgggcgattccgtgaagggcaggttcaccatcagccgcgacagggccaagaacacagtggacctgcagatggataatctggagccagaggacacagccgtgtactattgttccgccagatctcggggctacgtgctgtccgtgctgagaagcgtggactcctacgattattggggacagggcacccaggtgacagtgagcggcggaggaggcagcggaggaggaggatctggcggaggcggaagcatggcccaggtccagctggtggagagcggaggaggactggtgcaggctggaggctccctgaggctgtcttgcgctgctagcggcaggaccttctccaactacgctatgggctggtttcgccaggcccctggaaaggaaagagaatttgtggccgctatctcctggaccggcgtgtctacatactatgccgattctgtcaaaggcaggttcaccatcagcagagacaacgataagaatacagtgtatgtgcagatgaactccctgatccccgaggacaccgctatctactattgtgccgctgtgcgcgccaggtctttcagcgatacatactctcgggtgaatgagtacgactactggggccagggtacacaggtgacagtgatcctggattatagctttaccggaggagctggaagggacatccctccaccacagatcgaggaggcttgcgagctgccagagtgtcaggtggacgctggcaacaaggtgtgcaatctgcagtgtaacaatcacgcctgcggatgggacggaggcgattgtagcctgaacttcaatgacccatggaagaactgcacccagtctctgcagtgttggaagtactttagcgacggccactgcgattcccagtgtaactctgccggctgcctgttcgacggatttgattgtcagctgacagagggccagtgcaatcctctgtacgaccagtattgcaaggaccacttctctgatggccactgcgaccagggatgtaacagcgccgagtgtgagtgggacggcctggattgcgctgagcacgtgccagagcggctggctgctggaaccctggtgctggtggtgctgctgcctccagatcagctgagaaacaattccttccactttctgcgggagctgtctcacgtgctgcacacaaatgtggtgttcaagagagacgctcagggccagcagatgatctttccttactatggacacgaggaggagctgagaaagcaccccatcaagcggtccaccgtgggatgggccacaagctccctgctgccaggaacctctggaggccgccagaggagagagctggaccctatggacatcaggggctccatcgtgtacctggagatcgataacagacagtgcgtgcagtctagctcccagtgcttccagtctgctacagacgtggccgcttttctgggcgctctggcctctctgggaagcctgaatatcccatacaagatcgaggccgtgaagagcgagcctgtggagccacctctgccatcccagctgcacctgatgtatgtggccgctgccgctttcgtgctgctgttctttgtgggatgtggcgtgctgctgtccaggaagcggcgcaggcagctgtgcatccagaagctgatgaagctgctgtctagcatcgagcaggcttgcgacatctgtaggctgaagaagctgaagtgtagcaaggagaagcctaagtgcgccaagtgtctgaagaacaattgggagtgcagatattctccaaagaccaagcgcagccctctgaccagggctcacctgacagaggtggagtctagactggagcggctggagcagctgttcctgctgatctttccaagagaggacctggatatgatcctgaagatggatagcctgcaggacatcaaggccctgctgaccggcctgttcgtgcaggataacgtgaataaggatgctgtgacagacaggctggctagcgtggagaccgacatgcctctgacactgcgccagcacaggatctccgccacctcctctagcgaggagtcctctaacaagggacagaggcagctgacagtgagcgccgctgccggaggctccggaggctctggaggcagcgatgctctggacgatttcgacctggatatgctgggcagcgacgccctggacgattttgacctggacatgctcggcagcgacgcactcgatgactttgacctggacatgctgggctctgatgctctcgatgattttgacctggatatgctgggaagctgaggatcccccctgccctgaacatgtgtgcgcacacgtgcgtgctcttctgtcacccatgtgcctttaagcctatagcccacggacccccagaccaccctacccccagcctggttttgagctaagactgacgtacctcctcactccagaagatggacagagaactcaagacctgggggagggtgtgtattcacgggggtgaccccactatttgtcttatccctccagctcagtcctggccttcgtgtgtttttgtaagataaaccatttttaacacataccactctgttgtaaataagctgacgctactgtaaatacagaaaggaagaggttgagatgggggttgggaggaaggggtggggctcccaccagctgggcgagcctccaactcgagatctcttccgctctccttccatgtgtacataactgtcactcaagaaggtgattgacagattctgatttatatttgtgtattttcctggatttataggatgtgacttttctgattaatatatttaatatattgaataaaaaatagacatgtagttgaaattgagtctttttttctgtttttgttttttgtttttttttttttgtttttgtttttgtttttttgttttgtttttcgagacagggtttctctgtatagccctggctgtcctggagctcactttgtagaccaggctggcctcgaactcagaaatccgcctgcctctgcctcccgagtgctgggattaaaggcgtgcaccaccatgcctggctttttctgacagcactagacattttgccatgattatataagagacagcagtagccctgggcaaatcttagctgttgccagtgatctggtcagcctgggttacttacctgtaggtgataggtcatgatgaagcctgcttcatgcagccatttaggagaactctgggactagcttgcctttctcacacaaacacctgtctcaccatggtgcccggatggtttagacttgctgtgtagcttggctagtttcaagctgtcagtcttcctatctccacttcctgagtgttgggattatagatgttcaccctacacatgcatcgggagctagttcctaatgtgggaagcctctggttaccgctggctgccagacctcagtggacagcggctaacccagggactagagcagcaagatagacctgcggccgccaccgcggtggagctccagcttttgttccctttagtgagggttaattgcgcgcttggcgtaatcatggtcatagctgtttcctgtgtgaaattgttatccgctcacaattccacacaacatacgagccggaagcataaagtgtaaagcctggggtgcctaatgagtgagctaactcacattaattgcgttgcgctcactgcccgctttccagtcgggaaacctgtcgtgccagctgcattaatgaatcggccaacgcgcggggagaggcggtttgcgtattgggcgctcttccgcttcctcgctcactgactcgctgcgctcggtcgttcggctgcggcgagcggtatcagctcactcaaaggcggtaatacggttatccacagaatcaggggataacgcaggaaagaacatgtgagcaaaaggccagcaaaaggccaggaaccgtaaaaaggccgcgttgctggcgtttttccataggctccgcccccctgacgagcatcacaaaaatcgacgctcaagtcagaggtggcgaaacccgacaggactataaagataccaggcgtttccccctggaagctccctcgtgcgctctcctgttccgaccctgccgcttaccggatacctgtccgcctttctcccttcgggaagcgtggcgctttctcatagctcacgctgtaggtatctcagttcggtgtaggtcgttcgctccaagctgggctgtgtgcacgaaccccccgttcagcccgaccgctgcgccttatccggtaactatcgtcttgagtccaacccggtaagacacgacttatcgccactggcagcagccactggtaacaggattagcagagcgaggtatgtaggcggtgctacagagttcttgaagtggtggcctaactacggctacactagaaggacagtatttggtatctgcgctctgctgaagccagttaccttcggaaaaagagttggtagctcttgatccggcaaacaaaccaccgctggtagcggtggtttttttgtttgcaagcagcagattacgcgcagaaaaaaaggatctcaagaagatcctttgatcttttctacggggtctgacgctcagtggaacgaaaactcacgttaagggattttggtcatgagattatcaaaaaggatcttcacctagatccttttaaattaaaaatgaagttttaaatcaatctaaagtatatatgagtaaacttggtctgacagttaccaatgcttaatcagtgaggcacctatctcagcgatctgtctatttcgttcatccatagttgcctgactccccgtcgtgtagataactacgatacgggagggcttaccatctggccccagtgctgcaatgataccgcgagacccacgctcaccggctccagatttatcagcaataaaccagccagccggaagggccgagcgcagaagtggtcctgcaactttatccgcctccatccagtctattaattgttgccgggaagctagagtaagtagttcgccagttaatagtttgcgcaacgttgttgccattgctacaggcatcgtggtgtcacgctcgtcgtttggtatggcttcattcagctccggttcccaacgatcaaggcgagttacatgatcccccatgttgtgcaaaaaagcggttagctccttcggtcctccgatcgttgtcagaagtaagttggccgcagtgttatcactcatggttatggcagcactgcataattctcttactgtcatgccatccgtaagatgcttttctgtgactggtgagtactcaaccaagtcattctgagaatagtgtatgcggcgaccgagttgctcttgcccggcgtcaatacgggataataccgcgccacatagcagaactttaaaagtgctcatcattggaaaacgttcttcggggcgaaaactctcaaggatcttaccgctgttgagatccagttcgatgtaacccactcgtgcacccaactgatcttcagcatcttttactttcaccagcgtttctgggtgagcaaaaacaggaaggcaaaatgccgcaaaaaagggaataagggcgacacggaaatgttgaatactcatactcttcctttttcaatattattgaagcatttatcagggttattgtctcatgagcggatacatatttgaatgtatttagaaaaataaacaaataggggttccgcgcacatttccccgaaaagtgccac

SEQ ID NO: 12 - DNA, 8485 bp, synthetic construct
  source 1..8485: mol_type = other DNA
gagggcctatttcccatgattccttcatatttgcatatacgatacaaggctgttagagagataattggaattaatttgactgtaaacacaaagatattagtacaaaatacgtgacgtagaaagtaataatttcttgggtagtttgcagttttaaaattatgttttaaaatggactatcatatgcttaccgtaacttgaaagtatttcgatttcttggctttatatatcttgtggaaaggacgaaacaccgctccaggaccctcgtcggggttttagagctagaaatagcaagttaaaataaggctagtccgttatcaacttgaaaaagtggcaccgagtcggtgcttttttgttttagagctagaaatagcaagttaaaataaggctagtccgtttttagcgcgtgcgccaattctgcagacaaatggctctagaggtacccgttacataacttacggtaaatggcccgcctggctgaccgcccaacgacccccgcccattgacgtcaatagtaacgccaatagggactttccattgacgtcaatgggtggagtatttacggtaaactgcccacttggcagtacatcaagtgtatcatatgccaagtacgccccctattgacgtcaatgacggtaaatggcccgcctggcattgtgcccagtacatgaccttatgggactttcctacttggcagtacatctacgtattagtcatcgctattaccatggtcgaggtgagccccacgttctgcttcactctccccatctcccccccctccccacccccaattttgtatttatttattttttaattattttgtgcagcgatgggggcggggggggggggggggcggggcgaggggcggggcggggcgaggcggagaggtgcggcggcagccaatcagagcggcgcgctccgaaagtttccttttatggcgaggcggcggcggcggcggccctataaaaagcgaagcgcgcggcgggcgggagtcgctgcgcgctgccttcgccccgtgccccgctccgccgccgcctcgcgccgcccgccccggctctgactgaccgcgttactcccacaggtgagcgggcgggacggcccttctcctccgggctgtaattagctgagcaagaggtaagggtttaagggatggttggttggtggggtattaatgtttaattacctggagcacctgcctgaaatcactttttttcaggttggaccggtgccaccatggactataaggaccacgacggagactacaaggatcatgatattgattacaaagacgatgacgataagatggccccaaagaagaagcggaaggtcggtatccacggagtcccagcagccgacaagaagtacagcatcggcctggacatcggcaccaactctgtgggctgggccgtgatcaccgacgagtacaaggtgcccagcaagaaattcaaggtgctgggcaacaccgaccggcacagcatcaagaagaacctgatcggagccctgctgttcgacagcggcgaaacagccgaggccacccggctgaagagaaccgccagaagaagatacaccagacggaagaaccggatctgctatctgcaagagatcttcagcaacgagatggccaaggtggacgacagcttcttccacagactggaagagtccttcctggtggaagaggataagaagcacgagcggcaccccatcttcggcaacatcgtggacgaggtggcctaccacgagaagtaccccaccatctaccacctgagaaagaaactggtggacagcaccgacaaggccgacctgcggctgatctatctggccctggcccacatgatcaagttccggggccacttcctgatcgagggcgacctgaaccccgacaacagcgacgtggacaagctgttcatccagctggtgcagacctacaaccagctgttcgaggaaaaccccatcaacgccagcggcgtggacgccaaggccatcctgtctgccagactgagcaagagcagacggctggaaaatctgatcgcccagctgcccggcgagaagaagaatggcctgttcggaaacctgattgccctgagcctgggcctgacccccaacttcaagagcaacttcgacctggccgaggatgccaaactgcagctgagcaaggacacctacgacgacgacctggacaacctgctggcccagatcggcgaccagtacgccgacctgtttctggccgccaagaacctgtccgacgccatcctgctgagcgacatcctgagagtgaacaccgagatcaccaaggcccccctgagcgcctctatgatcaagagatacgacgagcaccaccaggacctgaccctgctgaaagctctcgtgcggcagcagctgcctgagaagtacaaagagattttcttcgaccagagcaagaacggctacgccggctacattgacggcggagccagccaggaagagttctacaagttcatcaagcccatcctggaaaagatggacggcaccgaggaactgctcgtgaagctgaacagagaggacctgctgcggaagcagcggaccttcgacaacggcagcatcccccaccagatccacctgggagagctgcacgccattctgcggcggcaggaagatttttacccattcctgaaggacaaccgggaaaagatcgagaagatcctgaccttccgcatcccctactacgtgggccctctggccaggggaaacagcagattcgcctggatgaccagaaagagcgaggaaaccatcaccccctggaacttcgaggaagtggtggacaagggcgcttccgcccagagcttcatcgagcggatgaccaacttcgataagaacctgcccaacgagaaggtgctgcccaagcacagcctgctgtacgagtacttcaccgtgtataacgagctgaccaaagtgaaatacgtgaccgagggaatgagaaagcccgccttcctgagcggcgagcagaaaaaggccatcgtggacctgctgttcaagaccaaccggaaagtgaccgtgaagcagctgaaagaggactacttcaagaaaatcgagtgcttcgactccgtggaaatctccggcgtggaagatcggttcaacgcctccctgggcacataccacgatctgctgaaaattatcaaggacaaggacttcctggacaatgaggaaaacgaggacattctggaagatatcgtgctgaccctgacactgtttgaggacagagagatgatcgaggaacggctgaaaacctatgcccacctgttcgacgacaaagtgatgaagcagctgaagcggcggagatacaccggctggggcaggctgagccggaagctgatcaacggcatccgggacaagcagtccggcaagacaatcctggatttcctgaagtccgacggcttcgccaacagaaacttcatgcagctgatccacgacgacagcctgacctttaaagaggacatccagaaagcccaggtgtccggccagggcgatagcctgcacgagcacattgccaatctggccggcagccccgccattaagaagggcatcctgcagacagtgaaggtggtggacgagctcgtgaaagtgatgggccggcacaagcccgagaacatcgtgatcgaaatggccagagagaaccagaccacccagaagggacagaagaacagccgcgagagaatgaagcggatcgaagagggcatcaaagagctgggcagccagatcctgaaagaacaccccgtggaaaacacccagctgcagaacgagaagctgtacctgtactacctgcagaatgggcgggatatgtacgtggaccaggaactggacatcaaccggctgtccgactacgatgtggaccatatcgtgcctcagagctttctgaaggacgactccatcgacaacaaggtgctgaccagaagcgacaagaaccggggcaagagcgacaacgtgccctccgaagaggtcgtgaagaagatgaagaactactggcggcagctgctgaacgccaagctgattacccagagaaagttcgacaatctgaccaaggccgagagaggcggcctgagcgaactggataaggccggcttcatcaagagacagctggtggaaacccggcagatcacaaagcacgtggcacagatcctggactcccggatgaacactaagtacgacgagaatgacaagctgatccgggaagtgaaagtgatcaccctgaagtccaagctggtgtccgatttccggaaggatttccagttttacaaagtgcgcgagatcaacaactaccaccacgcccacgacgcctacctgaacgccgtcgtgggaaccgccctgatcaaaaagtaccctaagctggaaagcgagttcgtgtacggcgactacaaggtgtacgacgtgcggaagatgatcgccaagagcgagcaggaaatcggcaaggctaccgccaagtacttcttctacagcaacatcatgaactttttcaagaccgagattaccctggccaacggcgagatccggaagcggcctctgatcgagacaaacggcgaaaccggggagatcgtgtgggataagggccgggattttgccaccgtgcggaaagtgctgagcatgccccaagtgaatatcgtgaaaaagaccgaggtgcagacaggcggcttcagcaaagagtctatcctgcccaagaggaacagcgataagctgatcgccagaaagaaggactgggaccctaagaagtacggcggcttcgacagccccaccgtggcctattctgtgctggtggtggccaaagtggaaaagggcaagtccaagaaactgaagagtgtgaaagagctgctggggatcaccatcatggaaagaagcagcttcgagaagaatcccatcgactttctggaagccaagggctacaaagaagtgaaaaaggacctgatcatcaagctgcctaagtactccctgttcgagctggaaaacggccggaagagaatgctggcctctgccggcgaactgcagaagggaaacgaactggccctgccctccaaatatgtgaacttcctgtacctggccagccactatgagaagctgaagggctcccccgaggataatgagcagaaacagctgtttgtggaacagcacaagcactacctggacgagatcatcgagcagatcagcgagttctccaagagagtgatcctggccgacgctaatctggacaaagtgctgtccgcctacaacaagcaccgggataagcccatcagagagcaggccgagaatatcatccacctgtttaccctgaccaatctgggagcccctgccgccttcaagtactttgacaccaccatcgaccggaagaggtacaccagcaccaaagaggtgctggacgccaccctgatccaccagagcatcaccggcctgtacgagacacggatcgacctgtctcagctgggaggcgacaaaaggccggcggccacgaaaaaggccggccaggcaaaaaagaaaaagtaagaattcctagagctcgctgatcagcctcgactgtgccttctagttgccagccatctgttgtttgcccctcccccgtgccttccttgaccctggaaggtgccactcccactgtcctttcctaataaaatgaggaaattgcatcgcattgtctgagtaggtgtcattctattctggggggtggggtggggcaggacagcaagggggaggattgggaagagaatagcaggcatgctggggagcggccgcaggaacccctagtgatggagttggccactccctctctgcgcgctcgctcgctcactgaggccgggcgaccaaaggtcgcccgacgcccgggctttgcccgggcggcctcagtgagcgagcgagcgcgcagctgcctgcaggggcgcctgatgcggtattttctccttacgcatctgtgcggtatttcacaccgcatacgtcaaagcaaccatagtacgcgccctgtagcggcgcattaagcgcggcgggtgtggtggttacgcgcagcgtgaccgctacacttgccagcgccttagcgcccgctcctttcgctttcttcccttcctttctcgccacgttcgccggctttccccgtcaagctctaaatcgggggctccctttagggttccgatttagtgctttacggcacctcgaccccaaaaaacttgatttgggtgatggttcacgtagtgggccatcgccctgatagacggtttttcgccctttgacgttggagtccacgttctttaatagtggactcttgttccaaactggaacaacactcaactctatctcgggctattcttttgatttataagggattttgccgatttcggtctattggttaaaaaatgagctgatttaacaaaaatttaacgcgaattttaacaaaatattaacgtttacaattttatggtgcactctcagtacaatctgctctgatgccgcatagttaagccagccccgacacccgccaacacccgctgacgcgccctgacgggcttgtctgctcccggcatccgcttacagacaagctgtgaccgtctccgggagctgcatgtgtcagaggttttcaccgtcatcaccgaaacgcgcgagacgaaagggcctcgtgatacgcctatttttataggttaatgtcatgataataatggtttcttagacgtcaggtggcacttttcggggaaatgtgcgcggaacccctatttgtttatttttctaaatacattcaaatatgtatccgctcatgagacaataaccctgataaatgcttcaataatattgaaaaaggaagagtatgagtattcaacatttccgtgtcgcccttattcccttttttgcggcattttgccttcctgtttttgctcacccagaaacgctggtgaaagtaaaagatgctgaagatcagttgggtgcacgagtgggttacatcgaactggatctcaacagcggtaagatccttgagagttttcgccccgaagaacgttttccaatgatgagcacttttaaagttctgctatgtggcgcggtattatcccgtattgacgccgggcaagagcaactcggtcgccgcatacactattctcagaatgacttggttgagtactcaccagtcacagaaaagcatcttacggatggcatgacagtaagagaattatgcagtgctgccataaccatgagtgataacactgcggccaacttacttctgacaacgatcggaggaccgaaggagctaaccgcttttttgcacaacatgggggatcatgtaactcgccttgatcgttgggaaccggagctgaatgaagccataccaaacgacgagcgtgacaccacgatgcctgtagcaatggcaacaacgttgcgcaaactattaactggcgaactacttactctagcttcccggcaacaattaatagactggatggaggcggataaagttgcaggaccacttctgcgctcggcccttccggctggctggtttattgctgataaatctggagccggtgagcgtggaagccgcggtatcattgcagcactggggccagatggtaagccctcccgtatcgtagttatctacacgacggggagtcaggcaactatggatgaacgaaatagacagatcgctgagataggtgcctcactgattaagcattggtaactgtcagaccaagtttactcatatatactttagattgatttaaaacttcatttttaatttaaaaggatctaggtgaagatcctttttgataatctcatgaccaaaatcccttaacgtgagttttcgttccactgagcgtcagaccccgtagaaaagatcaaaggatcttcttgagatcctttttttctgcgcgtaatctgctgcttgcaaacaaaaaaaccaccgctaccagcggtggtttgtttgccggatcaagagctaccaactctttttccgaaggtaactggcttcagcagagcgcagataccaaatactgttcttctagtgtagccgtagttaggccaccacttcaagaactctgtagcaccgcctacatacctcgctctgctaatcctgttaccagtggctgctgccagtggcgataagtcgtgtcttaccgggttggactcaagacgatagttaccggataaggcgcagcggtcgggctgaacggggggttcgtgcacacagcccagcttggagcgaacgacctacaccgaactgagatacctacagcgtgagctatgagaaagcgccacgcttcccgaagggagaaaggcggacaggtatccggtaagcggcagggtcggaacaggagagcgcacgagggagcttccagggggaaacgcctggtatctttatagtcctgtcgggtttcgccacctctgacttgagcgtcgatttttgtgatgctcgtcaggggggcggagcctatggaaaaacgccagcaacgcggcctttttacggttcctggccttttgctggccttttgctcacatg

SEQ ID NO: 13 - DNA, 5801 bp, synthetic construct
  source 1..5801: mol_type = other DNA
ctaaattgtaagcgttaatattttgttaaaattcgcgttaaatttttgttaaatcagctcattttttaaccaataggccgaaatcggcaaaatcccttataaatcaaaagaatagaccgagatagggttgagtgttgttccagtttggaacaagagtccactattaaagaacgtggactccaacgtcaaagggcgaaaaaccgtctatcagggcgatggcccactacgtgaaccatcaccctaatcaagttttttggggtcgaggtgccgtaaagcactaaatcggaaccctaaagggagcccccgatttagagcttgacggggaaagccggcgaacgtggcgagaaaggaagggaagaaagcgaaaggagcgggcgctagggcgctggcaagtgtagcggtcacgctgcgcgtaaccaccacacccgccgcgcttaatgcgccgctacagggcgcgtcccattcgccattcaggctgcgcaactgttgggaagggcgatcggtgcgggcctcttcgctattacgccagctggcgaaagggggatgtgctgcaaggcgattaagttgggtaacgccagggttttcccagtcacgacgttgtaaaacgacggccagtgagcgcgcgtaatacgactcactatagggcgaattgggtaccgggccccccctcgaggtcgacggtatcgataagcttgatatcgaattaatggcgtgttttggttggcgtaaggcgcctgtcagttaacggcagccggagtgcgcagccgccggcagcctcgctctgcccactgggtggggcgggaggtaggtggggtgaggcgagctggacgtgcgggcgcggtcggcctctggcggggcgggggaggggagggagggtcagcgaaagtagctcgcgcgcgagcggccgcccaccctccccttcctctgggggagtcgttttacccgccgccggccgggcctcgtcgtctgattggctctcggggcccagaaaactggcccttgccattggctcgtgttcgtgcaagttgagtccatccgccggccagcgggggcggcgaggaggcgctcccaggttccggccctcccctcggccccgcgccgcagagtctggccgcgcgcccctgcgcaacgtggcaggaagcgcgcgctgggggcggggacgggcagtagggctgagcggctgcggggcgggtgcaagcacgtttccgacttgagttgcctcaagaggggcgtgctgagccagacctccatcgcgcactccggggagtggagggaaggagcgagggctcagttgggctgttttggaggcaggaagcacttgctctcccaaagtcgctctgagttgttatcagtaagggagctgcagtggagtaggcggggagaaggccgcacccttctcctgaggagggaggggagtgttgcaatacctttctgggagttctctgctgcctcctggcttctgaggaccgccctgggcctgggagaatcccttccccctcttccctcgtgatctgcaactccagtcttatgcataaggagcactgtcctccgaacgggagcactgtcctccgaacgggagcactgtcctccgaacgggagcactgtcctccgaacgggagcactgtcctccgaacgggtaggcgtgtacggtgggaggcctatataagcagagctgaattcatggtgagcaagggcgaggaggataacatggccatcatcaaggagttcatgcgcttcaaggtgcacatggagggctccgtgaacggccacgagttcgagatcgagggcgagggcgagggccgcccctacgagggcacccagaccgccaagctgaaggtgaccaagggtggccccctgcccttcgcctgggacatcctgtcccctcagttcatgtacggctccaaggcctacgtgaagcaccccgccgacatccccgactacttgaagctgtccttccccgagggcttcaagtgggagcgcgtgatgaacttcgaggacggcggcgtggtgaccgtgacccaggactcctccctgcaggacggcgagttcatctacaaggtgaagctgcgcggcaccaacttcccctccgacggccccgtaatgcagaagaagaccatgggctgggaggcctcctccgagcggatgtaccccgaggacggcgccctgaagggcgagatcaagcagaggctgaagctgaaggacggcggccactacgacgctgaggtcaagaccacctacaaggccaagaagcccgtgcagctgcccggcgcctacaacgtcaacatcaagttggacatcacctcccacaacgaggactacaccatcgtggaacagtacgaacgcgccgagggccgccactccaccggcggcatggacgagctgtacaagtgagctagctcgacatgataagatacattgatgagtttggacaaaccacaactagaatgcagtgaaaaaaatgctttatttgtgaaatttgtgatgctattgctttatttgtgaaatttgtgatgctattgctttatttgtaaccattataagctgcaataaacaagttaacaacaacaattgcattcattttatgtttcaggttcagggggaggtgtgggaggttttttaaagcaagtaaaacctctacaaatgtggtagatccatttaaatgttaattaaaaacccgcttcggcgggtttttttatgagatgggcgggagtcttctgggcaggcttaaaggctaacctggtgtgtgggcgttgtcctgcaggggaattgaacaggtgtaaaattggagggacaagacttcccacagattttcggttttgtcgggaagttttttaataggggcaaataaggaaaatgggaggataggtagtcatctggggttttatgcagcaaaactacaggttattattgcttgtgatccgcctcggagtattttccatcgaggtagattaaagacatgctcacccgagttttatactctcctgcttgagatccttactacagtatgaaattacagtgtcgcgagttagactatgtaagcagaattttaatcatttttaaagagcccagtacttcatatccatttctcccgctccttctgcagccttatcaaaaggtattttagaacactcattttagccccattttcatttattatactggcttatccaacccctagacagagcattggcattttccctttcctgatcttagaagtctgatgactcatgaaaccagacagattagttacatacaccacaaatcgaggctgtagctggggcctcaacactgcagttcttttataactccttagtacactttttgttgatcctttgccttgatccttaattttcagtgtctatcacctctcccgtcaggtggtgttccacatttgggcctattctcagtccagggagttttacaacaatagatgtattgagaatccaacctaaagcttaactttccactcccatgaatgcctctctcctttttctccatttataaactgagctattaaccattaatggtttccaggtggatgtctccctgcagcccgggggatccactagttctagagcggccgccaccgcggtggagctccagcttttgttccctttagtgagggttaattgcgcgcttggcgtaatcatggtcatagctgtttcctgtgtgaaattgttatccgctcacaattccacacaacatacgagccggaagcataaagtgtaaagcctggggtgcctaatgagtgagctaactcacattaattgcgttgcgctcactgcccgctttccagtcgggaaacctgtcgtgccagctgcattaatgaatcggccaacgcgcggggagaggcggtttgcgtattgggcgctcttccgcttcctcgctcactgactcgctgcgctcggtcgttcggctgcggcgagcggtatcagctcactcaaaggcggtaatacggttatccacagaatcaggggataacgcaggaaagaacatgtgagcaaaaggccagcaaaaggccaggaaccgtaaaaaggccgcgttgctggcgtttttccataggctccgcccccctgacgagcatcacaaaaatcgacgctcaagtcagaggtggcgaaacccgacaggactataaagataccaggcgtttccccctggaagctccctcgtgcgctctcctgttccgaccctgccgcttaccggatacctgtccgcctttctcccttcgggaagcgtggcgctttctcatagctcacgctgtaggtatctcagttcggtgtaggtcgttcgctccaagctgggctgtgtgcacgaaccccccgttcagcccgaccgctgcgccttatccggtaactatcgtcttgagtccaacccggtaagacacgacttatcgccactggcagcagccactggtaacaggattagcagagcgaggtatgtaggcggtgctacagagttcttgaagtggtggcctaactacggctacactagaaggacagtatttggtatctgcgctctgctgaagccagttaccttcggaaaaagagttggtagctcttgatccggcaaacaaaccaccgctggtagcggtggtttttttgtttgcaagcagcagattacgcgcagaaaaaaaggatctcaagaagatcctttgatcttttctacggggtctgacgctcagtggaacgaaaactcacgttaagggattttggtcatgagattatcaaaaaggatcttcacctagatccttttaaattaaaaatgaagttttaaatcaatctaaagtatatatgagtaaacttggtctgacagttaccaatgcttaatcagtgaggcacctatctcagcgatctgtctatttcgttcatccatagttgcctgactccccgtcgtgtagataactacgatacgggagggcttaccatctggccccagtgctgcaatgataccgcgagacccacgctcaccggctccagatttatcagcaataaaccagccagccggaagggccgagcgcagaagtggtcctgcaactttatccgcctccatccagtctattaattgttgccgggaagctagagtaagtagttcgccagttaatagtttgcgcaacgttgttgccattgctacaggcatcgtggtgtcacgctcgtcgtttggtatggcttcattcagctccggttcccaacgatcaaggcgagttacatgatcccccatgttgtgcaaaaaagcggttagctccttcggtcctccgatcgttgtcagaagtaagttggccgcagtgttatcactcatggttatggcagcactgcataattctcttactgtcatgccatccgtaagatgcttttctgtgactggtgagtactcaaccaagtcattctgagaatagtgtatgcggcgaccgagttgctcttgcccggcgtcaatacgggataataccgcgccacatagcagaactttaaaagtgctcatcattggaaaacgttcttcggggcgaaaactctcaaggatcttaccgctgttgagatccagttcgatgtaacccactcgtgcacccaactgatcttcagcatcttttactttcaccagcgtttctgggtgagcaaaaacaggaaggcaaaatgccgcaaaaaagggaataagggcgacacggaaatgttgaatactcatactcttcctttttcaatattattgaagcatttatcagggttattgtctcatgagcggatacatatttgaatgtatttagaaaaataaacaaataggggttccgcgcacatttccccgaaaagtgccac

SEQ ID NO: 14 - DNA, 8486 bp, synthetic construct
  source 1..8486: mol_type = other DNA
gagggcctatttcccatgattccttcatatttgcatatacgatacaaggctgttagagagataattggaattaatttgactgtaaacacaaagatattagtacaaaatacgtgacgtagaaagtaataatttcttgggtagtttgcagttttaaaattatgttttaaaatggactatcatatgcttaccgtaacttgaaagtatttcgatttcttggctttatatatcttgtggaaaggacgaaacaccgggccgcacccttctccggagttttagagctagaaatagcaagttaaaataaggctagtccgttatcaacttgaaaaagtggcaccgagtcggtgcttttttgttttagagctagaaatagcaagttaaaataaggctagtccgtttttagcgcgtgcgccaattctgcagacaaatggctctagaggtacccgttacataacttacggtaaatggcccgcctggctgaccgcccaacgacccccgcccattgacgtcaatagtaacgccaatagggactttccattgacgtcaatgggtggagtatttacggtaaactgcccacttggcagtacatcaagtgtatcatatgccaagtacgccccctattgacgtcaatgacggtaaatggcccgcctggcattgtgcccagtacatgaccttatgggactttcctacttggcagtacatctacgtattagtcatcgctattaccatggtcgaggtgagccccacgttctgcttcactctccccatctcccccccctccccacccccaattttgtatttatttattttttaattattttgtgcagcgatgggggcggggggggggggggggcggggcgaggggcggggcggggcgaggcggagaggtgcggcggcagccaatcagagcggcgcgctccgaaagtttccttttatggcgaggcggcggcggcggcggccctataaaaagcgaagcgcgcggcgggcgggagtcgctgcgcgctgccttcgccccgtgccccgctccgccgccgcctcgcgccgcccgccccggctctgactgaccgcgttactcccacaggtgagcgggcgggacggcccttctcctccgggctgtaattagctgagcaagaggtaagggtttaagggatggttggttggtggggtattaatgtttaattacctggagcacctgcctgaaatcactttttttcaggttggaccggtgccaccatggactataaggaccacgacggagactacaaggatcatgatattgattacaaagacgatgacgataagatggccccaaagaagaagcggaaggtcggtatccacggagtcccagcagccgacaagaagtacagcatcggcctggacatcggcaccaactctgtgggctgggccgtgatcaccgacgagtacaaggtgcccagcaagaaattcaaggtgctgggcaacaccgaccggcacagcatcaagaagaacctgatcggagccctgctgttcgacagcggcgaaacagccgaggccacccggctgaagagaaccgccagaagaagatacaccagacggaagaaccggatctgctatctgcaagagatcttcagcaacgagatggccaaggtggacgacagcttcttccacagactggaagagtccttcctggtggaagaggataagaagcacgagcggcaccccatcttcggcaacatcgtggacgaggtggcctaccacgagaagtaccccaccatctaccacctgagaaagaaactggtggacagcaccgacaaggccgacctgcggctgatctatctggccctggcccacatgatcaagttccggggccacttcctgatcgagggcgacctgaaccccgacaacagcgacgtggacaagctgttcatccagctggtgcagacctacaaccagctgttcgaggaaaaccccatcaacgccagcggcgtggacgccaaggccatcctgtctgccagactgagcaagagcagacggctggaaaatctgatcgcccagctgcccggcgagaagaagaatggcctgttcggaaacctgattgccctgagcctgggcctgacccccaacttcaagagcaacttcgacctggccgaggatgccaaactgcagctgagcaaggacacctacgacgacgacctggacaacctgctggcccagatcggcgaccagtacgccgacctgtttctggccgccaagaacctgtccgacgccatcctgctgagcgacatcctgagagtgaacaccgagatcaccaaggcccccctgagcgcctctatgatcaagagatacgacgagcaccaccaggacctgaccctgctgaaagctctcgtgcggcagcagctgcctgagaagtacaaagagattttcttcgaccagagcaagaacggctacgccggctacattgacggcggagccagccaggaagagttctacaagttcatcaagcccatcctggaaaagatggacggcaccgaggaactgctcgtgaagctgaacagagaggacctgctgcggaagcagcggaccttcgacaacggcagcatcccccaccagatccacctgggagagctgcacgccattctgcggcggcaggaagatttttacccattcctgaaggacaaccgggaaaagatcgagaagatcctgaccttccgcatcccctactacgtgggccctctggccaggggaaacagcagattcgcctggatgaccagaaagagcgaggaaaccatcaccccctggaacttcgaggaagtggtggacaagggcgcttccgcccagagcttcatcgagcggatgaccaacttcgataagaacctgcccaacgagaaggtgctgcccaagcacagcctgctgtacgagtacttcaccgtgtataacgagctgaccaaagtgaaatacgtgaccgagggaatgagaaagcccgccttcctgagcggcgagcagaaaaaggccatcgtggacctgctgttcaagaccaaccggaaagtgaccgtgaagcagctgaaagaggactacttcaagaaaatcgagtgcttcgactccgtggaaatctccggcgtggaagatcggttcaacgcctccctgggcacataccacgatctgctgaaaattatcaaggacaaggacttcctggacaatgaggaaaacgaggacattctggaagatatcgtgctgaccctgacactgtttgaggacagagagatgatcgaggaacggctgaaaacctatgcccacctgttcgacgacaaagtgatgaagcagctgaagcggcggagatacaccggctggggcaggctgagccggaagctgatcaacggcatccgggacaagcagtccggcaagacaatcctggatttcctgaagtccgacggcttcgccaacagaaacttcatgcagctgatccacgacgacagcctgacctttaaagaggacatccagaaagcccaggtgtccggccagggcgatagcctgcacgagcacattgccaatctggccggcagccccgccattaagaagggcatcctgcagacagtgaaggtggtggacgagctcgtgaaagtgatgggccggcacaagcccgagaacatcgtgatcgaaatggccagagagaaccagaccacccagaagggacagaagaacagccgcgagagaatgaagcggatcgaagagggcatcaaagagctgggcagccagatcctgaaagaacaccccgtggaaaacacccagctgcagaacgagaagctgtacctgtactacctgcagaatgggcgggatatgtacgtggaccaggaactggacatcaaccggctgtccgactacgatgtggaccatatcgtgcctcagagctttctgaaggacgactccatcgacaacaaggtgctgaccagaagcgacaagaaccggggcaagagcgacaacgtgccctccgaagaggtcgtgaagaagatgaagaactactggcggcagctgctgaacgccaagctgattacccagagaaagttcgacaatctgaccaaggccgagagaggcggcctgagcgaactggataaggccggcttcatcaagagacagctggtggaaacccggcagatcacaaagcacgtggcacagatcctggactcccggatgaacactaagtacgacgagaatgacaagctgatccgggaagtgaaagtgatcaccctgaagtccaagctggtgtccgatttccggaaggatttccagttttacaaagtgcgcgagatcaacaactaccaccacgcccacgacgcctacctgaacgccgtcgtgggaaccgccctgatcaaaaagtaccctaagctggaaagcgagttcgtgtacggcgactacaaggtgtacgacgtgcggaagatgatcgccaagagcgagcaggaaatcggcaaggctaccgccaagtacttcttctacagcaacatcatgaactttttcaagaccgagattaccctggccaacggcgagatccggaagcggcctctgatcgagacaaacggcgaaaccggggagatcgtgtgggataagggccgggattttgccaccgtgcggaaagtgctgagcatgccccaagtgaatatcgtgaaaaagaccgaggtgcagacaggcggcttcagcaaagagtctatcctgcccaagaggaacagcgataagctgatcgccagaaagaaggactgggaccctaagaagtacggcggcttcgacagccccaccgtggcctattctgtgctggtggtggccaaagtggaaaagggcaagtccaagaaactgaagagtgtgaaagagctgctggggatcaccatcatggaaagaagcagcttcgagaagaatcccatcgactttctggaagccaagggctacaaagaagtgaaaaaggacctgatcatcaagctgcctaagtactccctgttcgagctggaaaacggccggaagagaatgctggcctctgccggcgaactgcagaagggaaacgaactggccctgccctccaaatatgtgaacttcctgtacctggccagccactatgagaagctgaagggctcccccgaggataatgagcagaaacagctgtttgtggaacagcacaagcactacctggacgagatcatcgagcagatcagcgagttctccaagagagtgatcctggccgacgctaatctggacaaagtgctgtccgcctacaacaagcaccgggataagcccatcagagagcaggccgagaatatcatccacctgtttaccctgaccaatctgggagcccctgccgccttcaagtactttgacaccaccatcgaccggaagaggtacaccagcaccaaagaggtgctggacgccaccctgatccaccagagcatcaccggcctgtacgagacacggatcgacctgtctcagctgggaggcgacaaaaggccggcggccacgaaaaaggccggccaggcaaaaaagaaaaagtaagaattcctagagctcgctgatcagcctcgactgtgccttctagttgccagccatctgttgtttgcccctcccccgtgccttccttgaccctggaaggtgccactcccactgtcctttcctaataaaatgaggaaattgcatcgcattgtctgagtaggtgtcattctattctggggggtggggtggggcaggacagcaagggggaggattgggaagagaatagcaggcatgctggggagcggccgcaggaacccctagtgatggagttggccactccctctctgcgcgctcgctcgctcactgaggccgggcgaccaaaggtcgcccgacgcccgggctttgcccgggcggcctcagtgagcgagcgagcgcgcagctgcctgcaggggcgcctgatgcggtattttctccttacgcatctgtgcggtatttcacaccgcatacgtcaaagcaaccatagtacgcgccctgtagcggcgcattaagcgcggcgggtgtggtggttacgcgcagcgtgaccgctacacttgccagcgccttagcgcccgctcctttcgctttcttcccttcctttctcgccacgttcgccggctttccccgtcaagctctaaatcgggggctccctttagggttccgatttagtgctttacggcacctcgaccccaaaaaacttgatttgggtgatggttcacgtagtgggccatcgccctgatagacggtttttcgccctttgacgttggagtccacgttctttaatagtggactcttgttccaaactggaacaacactcaactctatctcgggctattcttttgatttataagggattttgccgatttcggtctattggttaaaaaatgagctgatttaacaaaaatttaacgcgaattttaacaaaatattaacgtttacaattttatggtgcactctcagtacaatctgctctgatgccgcatagttaagccagccccgacacccgccaacacccgctgacgcgccctgacgggcttgtctgctcccggcatccgcttacagacaagctgtgaccgtctccgggagctgcatgtgtcagaggttttcaccgtcatcaccgaaacgcgcgagacgaaagggcctcgtgatacgcctatttttataggttaatgtcatgataataatggtttcttagacgtcaggtggcacttttcggggaaatgtgcgcggaacccctatttgtttatttttctaaatacattcaaatatgtatccgctcatgagacaataaccctgataaatgcttcaataatattgaaaaaggaagagtatgagtattcaacatttccgtgtcgcccttattcccttttttgcggcattttgccttcctgtttttgctcacccagaaacgctggtgaaagtaaaagatgctgaagatcagttgggtgcacgagtgggttacatcgaactggatctcaacagcggtaagatccttgagagttttcgccccgaagaacgttttccaatgatgagcacttttaaagttctgctatgtggcgcggtattatcccgtattgacgccgggcaagagcaactcggtcgccgcatacactattctcagaatgacttggttgagtactcaccagtcacagaaaagcatcttacggatggcatgacagtaagagaattatgcagtgctgccataaccatgagtgataacactgcggccaacttacttctgacaacgatcggaggaccgaaggagctaaccgcttttttgcacaacatgggggatcatgtaactcgccttgatcgttgggaaccggagctgaatgaagccataccaaacgacgagcgtgacaccacgatgcctgtagcaatggcaacaacgttgcgcaaactattaactggcgaactacttactctagcttcccggcaacaattaatagactggatggaggcggataaagttgcaggaccacttctgcgctcggcccttccggctggctggtttattgctgataaatctggagccggtgagcgtggaagccgcggtatcattgcagcactggggccagatggtaagccctcccgtatcgtagttatctacacgacggggagtcaggcaactatggatgaacgaaatagacagatcgctgagataggtgcctcactgattaagcattggtaactgtcagaccaagtttactcatatatactttagattgatttaaaacttcatttttaatttaaaaggatctaggtgaagatcctttttgataatctcatgaccaaaatcccttaacgtgagttttcgttccactgagcgtcagaccccgtagaaaagatcaaaggatcttcttgagatcctttttttctgcgcgtaatctgctgcttgcaaacaaaaaaaccaccgctaccagcggtggtttgtttgccggatcaagagctaccaactctttttccgaaggtaactggcttcagcagagcgcagataccaaatactgttcttctagtgtagccgtagttaggccaccacttcaagaactctgtagcaccgcctacatacctcgctctgctaatcctgttaccagtggctgctgccagtggcgataagtcgtgtcttaccgggttggactcaagacgatagttaccggataaggcgcagcggtcgggctgaacggggggttcgtgcacacagcccagcttggagcgaacgacctacaccgaactgagatacctacagcgtgagctatgagaaagcgccacgcttcccgaagggagaaaggcggacaggtatccggtaagcggcagggtcggaacaggagagcgcacgagggagcttccagggggaaacgcctggtatctttatagtcctgtcgggtttcgccacctctgacttgagcgtcgatttttgtgatgctcgtcaggggggcggagcctatggaaaaacgccagcaacgcggcctttttacggttcctggccttttgctggccttttgctcacatgt

SEQ ID NO: 15 - DNA, 8515 bp, synthetic construct
  source 1..8515: mol_type = other DNA
acgcgtgtagtcttatgcaatactcttgtagtcttgcaacatggtaacgatgagttagcaacatgccttacaaggagagaaaaagcaccgtgcatgccgattggtggaagtaaggtggtacgatcgtgccttattaggaaggcaacagacgggtctgacatggattggacgaaccactgaattgccgcattgcagagatattgtatttaagtgcctagctcgatacaataaacgggtctctctggttagaccagatctgagcctgggagctctctggctaactagggaacccactgcttaagcctcaataaagcttgccttgagtgcttcaagtagtgtgtgcccgtctgttgtgtgactctggtaactagagatccctcagacccttttagtcagtgtggaaaatctctagcagtggcgcccgaacagggacctgaaagcgaaagggaaaccagagctctctcgacgcaggactcggcttgctgaagcgcgcacggcaagaggcgaggggcggcgactggtgagtacgccaaaaattttgactagcggaggctagaaggagagagatgggtgcgagagcgtcagtattaagcgggggagaattagatcgcgatgggaaaaaattcggttaaggccagggggaaagaaaaaatataaattaaaacatatagtatgggcaagcagggagctagaacgattcgcagttaatcctggcctgttagaaacatcagaaggctgtagacaaatactgggacagctacaaccatcccttcagacaggatcagaagaacttagatcattatataatacagtagcaaccctctattgtgtgcatcaaaggatagagataaaagacaccaaggaagctttagacaagatagaggaagagcaaaacaaaagtaagaccaccgcacagcaagcggccactgatcttcagacctggaggaggagatatgagggacaattggagaagtgaattatataaatataaagtagtaaaaattgaaccattaggagtagcacccaccaaggcaaagagaagagtggtgcagagagaaaaaagagcagtgggaataggagctttgttccttgggttcttgggagcagcaggaagcactatgggcgcagcctcaatgacgctgacggtacaggccagacaattattgtctggtatagtgcagcagcagaacaatttgctgagggctattgaggcgcaacagcatctgttgcaactcacagtctggggcatcaagcagctccaggcaagaatcctggctgtggaaagatacctaaaggatcaacagctcctggggatttggggttgctctggaaaactcatttgcaccactgctgtgccttggaatgctagttggagtaataaatctctggaacagattggaatcacacgacctggatggagtgggacagagaaattaacaattacacaagcttaatacactccttaattgaagaatcgcaaaaccagcaagaaaagaatgaacaagaattattggaattagataaatgggcaagtttgtggaattggtttaacataacaaattggctgtggtatataaaattattcataatgatagtaggaggcttggtaggtttaagaatagtttttgctgtactttctatagtgaatagagttaggcagggatattcaccattatcgtttcagacccacctcccaaccccgaggggacccgacaggcccgaaggaatagaagaagaaggtggagagagagacagagacagatccattcgattagtgaacggatctcgacggttaacttttaaaagaaaaggggggattggggggtacagtgcaggggaaagaatagtagacataatagcaacagacatacaaactaaagaattacaaaaacaaattacaaaaattcaaaattttatcgacattgattattgactagttattaatagtaatcaattacggggtcattagttcatagcccatatatggagttccgcgttacataacttacggtaaatggcccgcctggctgaccgcccaacgacccccgcccattgacgtcaataatgacgtatgttcccatagtaacgccaatagggactttccattgacgtcaatgggtggagtatttacggtaaactgcccacttggcagtacatcaagtgtatcatatgccaagtacgccccctattgacgtcaatgacggtaaatggcccgcctggcattatgcccagtacatgaccttatgggactttcctacttggcagtacatctacgtattagtcatcgctattaccatggtcgaggtgagccccacgttctgcttcactctccccatctcccccccctccccacccccaattttgtatttatttattttttaattattttgtgcagcgatgggggcggggggggggggggggccccccccaggcggggcggggcggggcgaggggcggggcggggcgaggcggaaaggtgcggcggcagccaatcagagcggcgcgctccgaaagtttccttttatggcgaggcggcggcggcggcggccctataaaaagcgaagcgcgcggcgggcgggagtcgttgcgcgctgccttccccccgtgccccgctccgccgccgcctcgcgccgcccgccccggctctgactgaccgcgttactcccacaggtgagcgggcgggacggcccttctcctccgggctgtaattagcgcttggtttaatgacggcttgtttcttttctgtggctgcgtgaaagccttgaggggctccgggagggccctttgtgcggggggagcggctcggggggtgcgtgcgtgtgtgtgtgcgtggggagcgccgcgtgcggctccgcgctgcccggcggctgtgagcgctgcgggcgcggcgcggggctttgtgcgctccgcagtgtgcgcgaggggagcgcggccgggggcggtgccccgcggtgcggggggggctgcgaggggaacaaaggctgcgtgcggggtgtgtgcgtgggggggtgagcagggggtgtgggcgcgtcggtcgggctgcaaccccccctgcacccccctccccgagttgctgagcacggcccggcttcgggtgcggggctccgtacggggcgtggcgcggggctcgccgtgccgggcggggggtggcggcaggtgggggtgccgggcggggcggggccgcctcgggccggggagggctcgggggaaggggcgcggcggcccccggagcgccggcggctgtcgaggcgcggcgagccgcagccattgccttttatggtaatcgtgcgagagggcgcagggacttcctttgtcccaaatctgtgcggagccgaaatctgggaggcgccgccgcaccccctctagcgggcgcggggcgaagcggtgcggcgccggcaggaaggaaatgggcggggagggccttcgtgcgtcgccgcgccgccgtccccttctccctctccagcctcggggctgtccgcggggggacggctgccttcgggggggacggggcagggcggggttcggcttctggcgtgtgaccggcggctctagagcctctgctaaccatgttcatgccttcttctttttcctacagctcctgggcaacgtgctggttattgtgctgtctcatcattttggcaaagaattcgaatttaaatggatccgcggccgcatggagaccgacaccctgctgctgtgggtgctgctgctgtgggtgcccggcagcaccggcgacatggtgtcaaaaggcgaggagctgttcaccggcgtggtgcctatcctggtggagctggacggcgacgtgaacggccacaagttcagcgtgagcggagagggcgagggcgacgccacctacggcaagctgaccctgaagttcatctgcaccaccggcaagctgcctgtgccctggcctaccctggtgacaaccctgacctacggcgtgcagtgcttcagcagataccctgaccacatgaagcagcacgacttcttcaagagcgccatgcctgagggctacgtgcaggagagaaccatcttcttcaaggacgacggcaactacaagacaagagccgaggtgaagttcgagggcgacaccctggtgaacagaatcgagctgaagggcatcgacttcaaggaggacggcaacatcctgggccacaagctggagtacaactacaacagccacaacgtgtacatcatggccgacaagcagaagaacggcatcaaggtgaacttcaagatcagacacaacatcgaggacggcagcgtgcagctggccgaccactaccagcagaacaccccaatcggcgacggccctgtgctgctgcctgacaaccactacctgagcacccagagcgccctgagcaaggaccctaacgagaagagggaccacatggtgctgctggagttcgtgaccgccgccggcatcaccctgggcatggatgagctgtacaagaacgccgtgggccaggacacccaggaagtgatcgtggtgcctcacagcctgcctttcaaggtggtcgtgatcagcgccatcctggccctggtggtgctgaccatcatttctctgatcatcctgatcatgctgtggcagaagaagcctagggtcgacaatcaacctctggattacaaaatttgtgaaagattgactggtattcttaactatgttgctccttttacgctatgtggatacgctgctttaatgcctttgtatcatgctattgcttcccgtatggctttcattttctcctccttgtataaatcctggttgctgtctctttatgaggagttgtggcccgttgtcaggcaacgtggcgtggtgtgcactgtgtttgctgacgcaacccccactggttggggcattgccaccacctgtcagctcctttccgggactttcgctttccccctccctattgccacggcggaactcatcgccgcctgccttgcccgctgctggacaggggctcggctgttgggcactgacaattccgtggtgttgtcggggaaatcatcgtcctttccttggctgctcgcctgtgttgccacctggattctgcgcgggacgtccttctgctacgtcccttcggccctcaatccagcggaccttccttcccgcggcctgctgccggctctgcggcctcttccgcgtcttcgccttcgccctcagacgagtcggatctccctttgggccgcctccccgcctggtacctttaagaccaatgacttacaaggcagctgtagatcttagccactttttaaaagaaaaggggggactggaagggctaattcactcccaacgaaaataagatctgctttttgcttgtactgggtctctctggttagaccagatctgagcctgggagctctctggctaactagggaacccactgcttaagcctcaataaagcttgccttgagtgcttcaagtagtgtgtgcccgtctgttgtgtgactctggtaactagagatccctcagacccttttagtcagtgtggaaaatctctagcagtagtagttcatgtcatcttattattcagtatttataacttgcaaagaaatgaatatcagagagtgagaggaacttgtttattgcagcttataatggttacaaataaagcaatagcatcacaaatttcacaaataaagcatttttttcactgcattctagttgtggtttgtccaaactcatcaatgtatcttatcatgtctggctctagctatcccgcccctaactccgcccagttccgcccattctccgccccatggctgactaattttttttatttatgcagaggccgaggccgcctcggcctctgagctattccagaagtagtgaggaggcttttttggaggcctagacttttgcagagacggcccaaattcgtaatcatggtcatagctgtttcctgtgtgaaattgttatccgctcacaattccacacaacatacgagccggaagcataaagtgtaaagcctggggtgcctaatgagtgagctaactcacattaattgcgttgcgctcactgcccgctttccagtcgggaaacctgtcgtgccagctgcattaatgaatcggccaacgcgcggggagaggcggtttgcgtattgggcgctcttccgcttcctcgctcactgactcgctgcgctcggtcgttcggctgcggcgagcggtatcagctcactcaaaggcggtaatacggttatccacagaatcaggggataacgcaggaaagaacatgtgagcaaaaggccagcaaaaggccaggaaccgtaaaaaggccgcgttgctggcgtttttccataggctccgcccccctgacgagcatcacaaaaatcgacgctcaagtcagaggtggcgaaacccgacaggactataaagataccaggcgtttccccctggaagctccctcgtgcgctctcctgttccgaccctgccgcttaccggatacctgtccgcctttctcccttcgggaagcgtggcgctttctcatagctcacgctgtaggtatctcagttcggtgtaggtcgttcgctccaagctgggctgtgtgcacgaaccccccgttcagcccgaccgctgcgccttatccggtaactatcgtcttgagtccaacccggtaagacacgacttatcgccactggcagcagccactggtaacaggattagcagagcgaggtatgtaggcggtgctacagagttcttgaagtggtggcctaactacggctacactagaaggacagtatttggtatctgcgctctgctgaagccagttaccttcggaaaaagagttggtagctcttgatccggcaaacaaaccaccgctggtagcggtggtttttttgtttgcaagcagcagattacgcgcagaaaaaaaggatctcaagaagatcctttgatcttttctacggggtctgacgctcagtggaacgaaaactcacgttaagggattttggtcatgagattatcaaaaaggatcttcacctagatccttttaaattaaaaatgaagttttaaatcaatctaaagtatatatgagtaaacttggtctgacagttaccaatgcttaatcagtgaggcacctatctcagcgatctgtctatttcgttcatccatagttgcctgactccccgtcgtgtagataactacgatacgggagggcttaccatctggccccagtgctgcaatgataccgcgagacccacgctcaccggctccagatttatcagcaataaaccagccagccggaagggccgagcgcagaagtggtcctgcaactttatccgcctccatccagtctattaattgttgccgggaagctagagtaagtagttcgccagttaatagtttgcgcaacgttgttgccattgctacaggcatcgtggtgtcacgctcgtcgtttggtatggcttcattcagctccggttcccaacgatcaaggcgagttacatgatcccccatgttgtgcaaaaaagcggttagctccttcggtcctccgatcgttgtcagaagtaagttggccgcagtgttatcactcatggttatggcagcactgcataattctcttactgtcatgccatccgtaagatgcttttctgtgactggtgagtactcaaccaagtcattctgagaatagtgtatgcggcgaccgagttgctcttgcccggcgtcaatacgggataataccgcgccacatagcagaactttaaaagtgctcatcattggaaaacgttcttcggggcgaaaactctcaaggatcttaccgctgttgagatccagttcgatgtaacccactcgtgcacccaactgatcttcagcatcttttactttcaccagcgtttctgggtgagcaaaaacaggaaggcaaaatgccgcaaaaaagggaataagggcgacacggaaatgttgaatactcatactcttcctttttcaatattattgaagcatttatcagggttattgtctcatgagcggatacatatttgaatgtatttagaaaaataaacaaataggggttccgcgcacatttccccgaaaagtgccacctgacgtctaagaaaccattattatcatgacattaacctataaaaataggcgtatcacgaggccctttcgtctcgcgcgtttcggtgatgacggtgaaaacctctgacacatgcagctcccggagacggtcacagcttgtctgtaagcggatgccgggagcagacaagcccgtcagggcgcgtcagcgggtgttggcgggtgtcggggctggcttaactatgcggcatcagagcagattgtactgagagtgcaccatatgcggtgtgaaataccgcacagatgcgtaaggagaaaataccgcatcaggcgccattcgccattcaggctgcgcaactgttgggaagggcgatcggtgcgggcctcttcgctattacgccagctggcgaaagggggatgtgctgcaaggcgattaagttgggtaacgccagggttttcccagtcacgacgttgtaaaacgacggccagtgccaagctg

SEQ ID NO: 16 - DNA, 8694 bp, synthetic construct
  source 1..8694: mol_type = other DNA
acgcgtgtagtcttatgcaatactcttgtagtcttgcaacatggtaacgatgagttagcaacatgccttacaaggagagaaaaagcaccgtgcatgccgattggtggaagtaaggtggtacgatcgtgccttattaggaaggcaacagacgggtctgacatggattggacgaaccactgaattgccgcattgcagagatattgtatttaagtgcctagctcgatacaataaacgggtctctctggttagaccagatctgagcctgggagctctctggctaactagggaacccactgcttaagcctcaataaagcttgccttgagtgcttcaagtagtgtgtgcccgtctgttgtgtgactctggtaactagagatccctcagacccttttagtcagtgtggaaaatctctagcagtggcgcccgaacagggacctgaaagcgaaagggaaaccagagctctctcgacgcaggactcggcttgctgaagcgcgcacggcaagaggcgaggggcggcgactggtgagtacgccaaaaattttgactagcggaggctagaaggagagagatgggtgcgagagcgtcagtattaagcgggggagaattagatcgcgatgggaaaaaattcggttaaggccagggggaaagaaaaaatataaattaaaacatatagtatgggcaagcagggagctagaacgattcgcagttaatcctggcctgttagaaacatcagaaggctgtagacaaatactgggacagctacaaccatcccttcagacaggatcagaagaacttagatcattatataatacagtagcaaccctctattgtgtgcatcaaaggatagagataaaagacaccaaggaagctttagacaagatagaggaagagcaaaacaaaagtaagaccaccgcacagcaagcggccactgatcttcagacctggaggaggagatatgagggacaattggagaagtgaattatataaatataaagtagtaaaaattgaaccattaggagtagcacccaccaaggcaaagagaagagtggtgcagagagaaaaaagagcagtgggaataggagctttgttccttgggttcttgggagcagcaggaagcactatgggcgcagcctcaatgacgctgacggtacaggccagacaattattgtctggtatagtgcagcagcagaacaatttgctgagggctattgaggcgcaacagcatctgttgcaactcacagtctggggcatcaagcagctccaggcaagaatcctggctgtggaaagatacctaaaggatcaacagctcctggggatttggggttgctctggaaaactcatttgcaccactgctgtgccttggaatgctagttggagtaataaatctctggaacagattggaatcacacgacctggatggagtgggacagagaaattaacaattacacaagcttaatacactccttaattgaagaatcgcaaaaccagcaagaaaagaatgaacaagaattattggaattagataaatgggcaagtttgtggaattggtttaacataacaaattggctgtggtatataaaattattcataatgatagtaggaggcttggtaggtttaagaatagtttttgctgtactttctatagtgaatagagttaggcagggatattcaccattatcgtttcagacccacctcccaaccccgaggggacccgacaggcccgaaggaatagaagaagaaggtggagagagagacagagacagatccattcgattagtgaacggatctcgacggttaacttttaaaagaaaaggggggattggggggtacagtgcaggggaaagaatagtagacataatagcaacagacatacaaactaaagaattacaaaaacaaattacaaaaattcaaaattttatcgacattgattattgactagttattaatagtaatcaattacggggtcattagttcatagcccatatatggagttccgcgttacataacttacggtaaatggcccgcctggctgaccgcccaacgacccccgcccattgacgtcaataatgacgtatgttcccatagtaacgccaatagggactttccattgacgtcaatgggtggagtatttacggtaaactgcccacttggcagtacatcaagtgtatcatatgccaagtacgccccctattgacgtcaatgacggtaaatggcccgcctggcattatgcccagtacatgaccttatgggactttcctacttggcagtacatctacgtattagtcatcgctattaccatggtcgaggtgagccccacgttctgcttcactctccccatctcccccccctccccacccccaattttgtatttatttattttttaattattttgtgcagcgatgggggcggggggggggggggggccccccccaggcggggcggggcggggcgaggggcggggcggggcgaggcggaaaggtgcggcggcagccaatcagagcggcgcgctccgaaagtttccttttatggcgaggcggcggcggcggcggccctataaaaagcgaagcgcgcggcgggcgggagtcgttgcgcgctgccttccccccgtgccccgctccgccgccgcctcgcgccgcccgccccggctctgactgaccgcgttactcccacaggtgagcgggcgggacggcccttctcctccgggctgtaattagcgcttggtttaatgacggcttgtttcttttctgtggctgcgtgaaagccttgaggggctccgggagggccctttgtgcggggggagcggctcggggggtgcgtgcgtgtgtgtgtgcgtggggagcgccgcgtgcggctccgcgctgcccggcggctgtgagcgctgcgggcgcggcgcggggctttgtgcgctccgcagtgtgcgcgaggggagcgcggccgggggcggtgccccgcggtgcggggggggctgcgaggggaacaaaggctgcgtgcggggtgtgtgcgtgggggggtgagcagggggtgtgggcgcgtcggtcgggctgcaaccccccctgcacccccctccccgagttgctgagcacggcccggcttcgggtgcggggctccgtacggggcgtggcgcggggctcgccgtgccgggcggggggtggcggcaggtgggggtgccgggcggggcggggccgcctcgggccggggagggctcgggggaaggggcgcggcggcccccggagcgccggcggctgtcgaggcgcggcgagccgcagccattgccttttatggtaatcgtgcgagagggcgcagggacttcctttgtcccaaatctgtgcggagccgaaatctgggaggcgccgccgcaccccctctagcgggcgcggggcgaagcggtgcggcgccggcaggaaggaaatgggcggggagggccttcgtgcgtcgccgcgccgccgtccccttctccctctccagcctcggggctgtccgcggggggacggctgccttcgggggggacggggcagggcggggttcggcttctggcgtgtgaccggcggctctagagcctctgctaaccatgttcatgccttcttctttttcctacagctcctgggcaacgtgctggttattgtgctgtctcatcattttggcaaagaattcgaatttaaatggatccgcggccgctggagaccgataccctgctgctgtgggtgctgctgctgtgggtgcctggctccaccggcgactacccatatgacgtccctgactatgcaggcgcccagcctgctagacctgaagagcctctggtagtgaaggttgaggaaggcgataatgccgtgctgcagtgcctgaagggcaccagcgacggccctactcagcagctgacctggagcagagagagcccactgaaacctttccttaaactgtccctgggcctgcccggcctgggcatccacatgcggcccctggccatctggctgttcatcttcaacgtgagccagcagatgggaggcttctacctgtgccagcctggccctcctagcgagaaggcctggcagccaggctggaccgtgaacgtggagggcagcggcgagctgttcaggtggaacgtgtctgacctgggcggcctggggtgcggcctgaagaacaggagcagcgagggcccttcctccccttccggaaagctgatgagcccaaagctgtacgtgtgggccaaggacagacctgagatctgggagggcgagcctccttgtctgccacctagggatagcctgaaccagagcctgagccaggacctgaccatggcccctggcagcaccctgtggctgagctgcggcgtgcctcctgacagcgtgagcagagggcctctgagctggacccacgtgcaccctaagggccctaagtccctgctgagcttagaactgaaggacgacaggcccgccagggacatgtgggtcatggagaccggcctgctgctgcctagggccaccgcccaggacgccggcaagtactactgtcataggggaaatctgactatgagcttccacttagaaataaccgctagacctgtgctttggcattggctgctgagaacaggaggatggaaggtggacgaacagaagctgatcagcgaggaggacctgaatgccgtgggccaggacacacaggaagtgatcgtggtgccccatagcctgccttttaaggtggttgtgatctccgctattctggcactggtggtgctgacaatcattagcctgatcatcctgatcatgctgtggcagaagaagcctagagtcgacaatcaacctctggattacaaaatttgtgaaagattgactggtattcttaactatgttgctccttttacgctatgtggatacgctgctttaatgcctttgtatcatgctattgcttcccgtatggctttcattttctcctccttgtataaatcctggttgctgtctctttatgaggagttgtggcccgttgtcaggcaacgtggcgtggtgtgcactgtgtttgctgacgcaacccccactggttggggcattgccaccacctgtcagctcctttccgggactttcgctttccccctccctattgccacggcggaactcatcgccgcctgccttgcccgctgctggacaggggctcggctgttgggcactgacaattccgtggtgttgtcggggaaatcatcgtcctttccttggctgctcgcctgtgttgccacctggattctgcgcgggacgtccttctgctacgtcccttcggccctcaatccagcggaccttccttcccgcggcctgctgccggctctgcggcctcttccgcgtcttcgccttcgccctcagacgagtcggatctccctttgggccgcctccccgcctggtacctttaagaccaatgacttacaaggcagctgtagatcttagccactttttaaaagaaaaggggggactggaagggctaattcactcccaacgaaaataagatctgctttttgcttgtactgggtctctctggttagaccagatctgagcctgggagctctctggctaactagggaacccactgcttaagcctcaataaagcttgccttgagtgcttcaagtagtgtgtgcccgtctgttgtgtgactctggtaactagagatccctcagacccttttagtcagtgtggaaaatctctagcagtagtagttcatgtcatcttattattcagtatttataacttgcaaagaaatgaatatcagagagtgagaggaacttgtttattgcagcttataatggttacaaataaagcaatagcatcacaaatttcacaaataaagcatttttttcactgcattctagttgtggtttgtccaaactcatcaatgtatcttatcatgtctggctctagctatcccgcccctaactccgcccagttccgcccattctccgccccatggctgactaattttttttatttatgcagaggccgaggccgcctcggcctctgagctattccagaagtagtgaggaggcttttttggaggcctagacttttgcagagacggcccaaattcgtaatcatggtcatagctgtttcctgtgtgaaattgttatccgctcacaattccacacaacatacgagccggaagcataaagtgtaaagcctggggtgcctaatgagtgagctaactcacattaattgcgttgcgctcactgcccgctttccagtcgggaaacctgtcgtgccagctgcattaatgaatcggccaacgcgcggggagaggcggtttgcgtattgggcgctcttccgcttcctcgctcactgactcgctgcgctcggtcgttcggctgcggcgagcggtatcagctcactcaaaggcggtaatacggttatccacagaatcaggggataacgcaggaaagaacatgtgagcaaaaggccagcaaaaggccaggaaccgtaaaaaggccgcgttgctggcgtttttccataggctccgcccccctgacgagcatcacaaaaatcgacgctcaagtcagaggtggcgaaacccgacaggactataaagataccaggcgtttccccctggaagctccctcgtgcgctctcctgttccgaccctgccgcttaccggatacctgtccgcctttctcccttcgggaagcgtggcgctttctcatagctcacgctgtaggtatctcagttcggtgtaggtcgttcgctccaagctgggctgtgtgcacgaaccccccgttcagcccgaccgctgcgccttatccggtaactatcgtcttgagtccaacccggtaagacacgacttatcgccactggcagcagccactggtaacaggattagcagagcgaggtatgtaggcggtgctacagagttcttgaagtggtggcctaactacggctacactagaaggacagtatttggtatctgcgctctgctgaagccagttaccttcggaaaaagagttggtagctcttgatccggcaaacaaaccaccgctggtagcggtggtttttttgtttgcaagcagcagattacgcgcagaaaaaaaggatctcaagaagatcctttgatcttttctacggggtctgacgctcagtggaacgaaaactcacgttaagggattttggtcatgagattatcaaaaaggatcttcacctagatccttttaaattaaaaatgaagttttaaatcaatctaaagtatatatgagtaaacttggtctgacagttaccaatgcttaatcagtgaggcacctatctcagcgatctgtctatttcgttcatccatagttgcctgactccccgtcgtgtagataactacgatacgggagggcttaccatctggccccagtgctgcaatgataccgcgagacccacgctcaccggctccagatttatcagcaataaaccagccagccggaagggccgagcgcagaagtggtcctgcaactttatccgcctccatccagtctattaattgttgccgggaagctagagtaagtagttcgccagttaatagtttgcgcaacgttgttgccattgctacaggcatcgtggtgtcacgctcgtcgtttggtatggcttcattcagctccggttcccaacgatcaaggcgagttacatgatcccccatgttgtgcaaaaaagcggttagctccttcggtcctccgatcgttgtcagaagtaagttggccgcagtgttatcactcatggttatggcagcactgcataattctcttactgtcatgccatccgtaagatgcttttctgtgactggtgagtactcaaccaagtcattctgagaatagtgtatgcggcgaccgagttgctcttgcccggcgtcaatacgggataataccgcgccacatagcagaactttaaaagtgctcatcattggaaaacgttcttcggggcgaaaactctcaaggatcttaccgctgttgagatccagttcgatgtaacccactcgtgcacccaactgatcttcagcatcttttactttcaccagcgtttctgggtgagcaaaaacaggaaggcaaaatgccgcaaaaaagggaataagggcgacacggaaatgttgaatactcatactcttcctttttcaatattattgaagcatttatcagggttattgtctcatgagcggatacatatttgaatgtatttagaaaaataaacaaataggggttccgcgcacatttccccgaaaagtgccacctgacgtctaagaaaccattattatcatgacattaacctataaaaataggcgtatcacgaggccctttcgtctcgcgcgtttcggtgatgacggtgaaaacctctgacacatgcagctcccggagacggtcacagcttgtctgtaagcggatgccgggagcagacaagcccgtcagggcgcgtcagcgggtgttggcgggtgtcggggctggcttaactatgcggcatcagagcagattgtactgagagtgcaccatatgcggtgtgaaataccgcacagatgcgtaaggagaaaataccgcatcaggcgccattcgccattcaggctgcgcaactgttgggaagggcgatcggtgcgggcctcttcgctattacgccagctggcgaaagggggatgtgctgcaaggcgattaagttgggtaacgccagggttttcccagtcacgacgttgtaaaacgacggccagtgccaagctg